European Patent Application EP 4 628 584 A1, published October 8, 2025. Title: Y CHROSOMAL GENES FOR THE TREATMENT OR DIAGNOSIS OF CARDIOVASCULAR DISEASE. Applicant: Johann Wolfgang Goethe-Universität Frankfurt am Main. Application EP. The sequence listing filed with the application follows.

SEQUENCE LISTING (53 sequences)

SEQ ID NO: 1 - protein, 263 aa, Homo sapiens
MARGPKKHLKRVAAPKHWMLDKLTGVFAPRPSTGPHKLRECLPLIVFLRNRLKYALTGDEVKKICMQRFIKIDGKVRVDVTYPAGFMDVISIEKTGEHFRLVYDTKGRFAVHRITVEEAKYKLCKVRKITVGVKGIPHLVTHDARTIRYPDPVIKVNDTVQIDLGTGKIINFIKFDTGNLCMVIGGANLGRVGVITNRERHPGSFDVVHVKDANGNSFATRLSNIFVIGNGNKPWISLPRGKGIRLTVAEERDKRLATKQSSG

SEQ ID NO: 2 - RNA, 870 nt, Homo sapiens
  source 1..870: mol_type = mRNA
cagagtttcgccatggcccggggccccaagaagcacttaaagcgtgttgcagcgccgaagcattggatgcttgacaaactaacgggtgtatttgcacctcgtccatcgacaggtccccacaagctgagggaatgtcttcctctgatcgtcttcctcaggaatagactcaagtatgcgttgactggagatgaggtaaagaagatatgtatgcaacgtttcatcaaaattgatggcaaggttcgagtggatgtcacataccctgctggattcatggatgtcatcagcatcgagaagacaggtgaacatttccgcctggtctatgacaccaagggccgttttgctgttcaccgcatcacagtggaagaggcaaagtacaagttgtgcaaagtgaggaagattactgtgggagtgaagggaatccctcacctggtgactcatgatgctcgaaccatccgctacccagatcctgtcatcaaggtgaacgatactgtgcagattgatttagggactggcaagataatcaactttatcaaatttgatacaggcaatttgtgtatggtgattggtggagccaacctcggtcgtgttggtgtgatcaccaacagggaaagacatcctggttcttttgatgtggtgcatgtgaaggatgccaatggcaacagctttgccacgaggctttccaacatttttgtcattggcaatggcaataaaccttggatttccctgcccaggggaaagggcattcgacttactgttgctgaagagagagataagaggctggccaccaaacagagcagtggctaaattgcagtagcagcatatctttttttctttgcacaaataaacagtgaattctcgttaaaaaaaaaa

SEQ ID NO: 3 - protein, 660 aa, Homo sapiens
MSHVVVKNDPELDQQLANLDLNSEKQSGGASTASKGRYIPPHLRNREASKGFHDKDSSGWSCSKDKDAYSSFGSRDSRGKPGYFSERGSGSRGRFDDRGRSDYDGIGNRERPGFGRFERSGHSRWCDKSVEDDWSKPLPPSERLEQELFSGGNTGINFEKYDDIPVEATGSNCPPHIENFSDIDMGEIIMGNIELTRYTRPTPVQKHAIPIIKGKRDLMACAQTGSGKTAAFLLPILSQIYTDGPGEALKAVKENGRYGRRKQYPISLVLAPTRELAVQIYEEARKFSYRSRVRPCVVYGGADIGQQIRDLERGCHLLVATPGRLVDMMERGKIGLDFCKYLVLDEADRMLDMGFEPQIRRIVEQDTMPPKGVRHTMMFSATFPKEIQMLARDFLDEYIFLAVGRVGSTSENITQKVVWVEDLDKRSFLLDILGATGSDSLTLVFVETKKGADSLEDFLYHEGYACTSIHGDRSQRDREEALHQFRSGKSPILVATAVAARGLDISNVRHVINFDLPSDIEEYVHRIGRTGRVGNLGLATSFFNEKNMNITKDLLDLLVEAKQEVPSWLENMAYEHHYKGGSRGRSKSNRFSGGFGARDYRQSSGSSSSGFGASRGSSSRSGGGGYGNSRGFGGGGYGGFYNSDGYGGNYNSQGVDWWGN

SEQ ID NO: 4 - RNA, 2319 nt, Homo sapiens
  source 1..2319: mol_type = mRNA
ccagtgtaagagttccgctattcggtctcacacctacagtggactacccgatttttcgcttctcttcagggatgagtcatgtggtggtgaaaaatgaccctgaactggaccagcagcttgctaatctggacctgaactctgaaaaacagagtggaggagcaagtacagcgagcaaagggcgctatatacctcctcacttaaggaacaaagaagcatctaaaggattccatgataaagacagttcaggttggagttgcagcaaagataaggatgcatatagcagttttgggtctcgagattctagaggaaagcctggttatttcagtgaacgtggaagtggatcaaggggaagatttgatgatcgtggacggagtgactatgatggtattggcaatcgtgaaagacctggctttggcagatttgaacggagtggacatagtcgttggtgtgacaagtcagttgaagatgattggtcaaaaccacttccaccaagtgaacgcttggagcaagaactgttttctggaggaaacacggggattaactttgagaaatatgatgatataccagtagaggcaaccggcagtaactgtcctccacatattgagaattttagcgatattgacatgggagaaattatcatggggaacattgaacttactcgctatactcgtcctactccagtgcaaaaacatgccattcctattattaagggaaaaagagacttagtggcttgtgcccaaacaggatctgggaaaactgcagcatttcttttacccatactgagtcagatatatacagatggtccaggagaagctttgaaggctgtgaaggaaaatggaaggtatgggcgccgcaaacaatatccaatatccttggttttagccccaacaagagaattggctgtacagatctatgaggaagccagaaaattttcctaccgatctagagttcgtccttgtgtagtttatggtggtgctgatattggtcagcagattcgggacttagaacgtggatgccacttgttagtagccactccaggacgtctagtggatatgatggaaagaggaaagattggattagacttctgcaagtacttagtgttggatgaagctgataggatgctggatatgggatttgaacctcagatacgtcgtatagttgaacaagatactatgccaccaaagggcgttcgtcacaccatgatgtttagtgctacttttcctaaggaaatacagatgcttgctcgtgactttttggatgaatatatctttttggctgtaggcagagtaggctctacctctgagaacatcacacagaaagtagtttgggtggaagacttagataaacggtcatttctactggacattttaggtgcaacagggagtgattcacttactttagtgtttgtggagaccaaaaagggagcagattccctggaggatttcttataccatgaaggatatgcttgtactagtattcatggagaccggtcacagagagatcgagaggaggcccttcaccagtttcgctcaggaaaaagcccaattctagtggctacagctgtggcagcacgaggactagacatttcaaatgtgagacatgttatcaattttgatttgccaagtgatattgaagaatatgtgcatcgtattggccgtacaggacgtgtaggaaacctgggccttgccacctcattctttaatgaaaaaaatatgaatattacaaaggatttgttggatcttcttgtagaagctaaacaagaagtgccttcttggttggaaaatatggcttatgaacaccactacaagggtggcagtcgtggacgatctaaaagtaatagattcagtggaggatttggtgccagagactatcgacaaagtagtggttccagcagttccggctttggtgctagtcgcggaagcagcagccgcagtggtggaggtggttacggcgacagcagaggatttggtggaggtggctatggaggcttctacaatagtgatggatatggaggaaattataactcccagggggttgactggtggggcaactgaatctgctttgcagcaaagtcacccttacaaagaagctaatatggaaaccacatgtaacttagccagactatattgtgtagcttcaagaacttgcagtacattaccagctgtgattctcctgataattcaagggagctcaaagtcacaagaagaaaaatgaaaggaaaaaacagcagccctattcagaaattggtttgaagatgtaattgctctagtttggattaaactcttcccctcctgctttagtgccaccccaaaaaaaaaa

SEQ ID NO: 5 - RNA, 4416 nt, Homo sapiens
  source 1..4416: mol_type = mRNA
ccagtgtaagagttccgctattcggtctcacacctacagtggactacccgatttttcgcttctcttcagggatgagtcatgtggtggtgaaaaatgaccctgaactggaccagcagcttgctaatctggacctgaactctgaaaaacagagtggaggagcaagtacagcgagcaaagggcgctatatacctcctcacttaaggaacaaagaagcatctaaaggattccatgataaagacagttcaggttggagttgcagcaaagataaggatgcatatagcagttttgggtctcgagattctagaggaaagcctggttatttcagtgaacgtggaagtggatcaaggggaagatttgatgatcgtggacggagtgactatgatggtattggcaatcgtgaaagacctggctttggcagatttgaacggagtggacatagtcgttggtgtgacaagtcagttgaagatgattggtcaaaaccacttccaccaagtgaacgcttggagcaagaactgttttctggaggaaacacggggattaactttgagaaatatgatgatataccagtagaggcaaccggcagtaactgtcctccacatattgagaattttagcgatattgacatgggagaaattatcatggggaacattgaacttactcgctatactcgtcctactccagtgcaaaaacatgccattcctattattaagggaaaaagagacttagtggcttgtgcccaaacaggatctgggaaaactgcagcatttcttttacccatactgagtcagatatatacagatggtccaggagaagctttgaaggctgtgaaggaaaatggaaggtatgggcgccgcaaacaatatccaatatccttggttttagccccaacaagagaattggctgtacagatctatgaggaagccagaaaattttcctaccgatctagagttcgtccttgtgtagtttatggtggtgctgatattggtcagcagattcgggacttagaacgtggatgccacttgttagtagccactccaggacgtctagtggatatgatggaaagaggaaagattggattagacttctgcaagtacttagtgttggatgaagctgataggatgctggatatgggatttgaacctcagatacgtcgtatagttgaacaagatactatgccaccaaagggcgttcgtcacaccatgatgtttagtgctacttttcctaaggaaatacagatgcttgctcgtgactttttggatgaatatatctttttggctgtaggcagagtaggctctacctctgagaacatcacacagaaagtagtttgggtggaagacttagataaacggtcatttctactggacattttaggtgcaacagggagtgattcacttactttagtgtttgtggagaccaaaaagggagcagattccctggaggatttcttataccatgaaggatatgcttgtactagtattcatggagaccggtcacagagagatcgagaggaggcccttcaccagtttcgctcaggaaaaagcccaattctagtggctacagctgtggcagcacgaggactagacatttcaaatgtgagacatgttatcaattttgatttgccaagtgatattgaagaatatgtgcatcgtattggccgtacaggacgtgtaggaaacctgggccttgccacctcattctttaatgaaaaaaatatgaatattacaaaggatttgttggatcttcttgtagaagctaaacaagaagtgccttcttggttggaaaatatggcttatgaacaccactacaagggtggcagtcgtggacgatctaaaagtaatagattcagtggaggatttggtgccagagactatcgacaaagtagtggttccagcagttccggctttggtgctagtcgcggaagcagcagccgcagtggtggaggtggttacggcgacagcagaggatttggtggaggtggctatggaggcttctacaatagtgatggatatggaggaaattataactcccagggggttgactggtggggcaactgaatctgctttgcagcaaagtcacccttacaaagaagctaatatggaaaccacatgtaacttagccagactatattgtgtagcttcaagaacttgcagtacattaccagctgtgattctcctgataattcaagggagctcaaagtcacaagaagaaaaatgaaaggaaaaaacagcagccctattcagaaattggtttgaagatgtaattgctctagtttggattaaactcttcccctcctgctttagtgccaccccaaactgcatttataattttgtgactgaggatcgtttgtttgttaacgtactgtgactttaactttagacaacttactactttgatgtcctgttggctcagtaatgctcacgataccaattgttttgacaaaataaatttactaaacttggcctaaaatcaaaccttggcacagaggtatgatacaactttaacaggagtcatcaattcatccataaatataaaaagggaaaaaaacttaaggcagtagtctgcattaggactgtttgagttttgcagacttggggttgggagaacatcttaaagcattaaagcatagttttttgtatggccaaccttactaaattaagttctgacttgctcactctatcctggataggcacttgggaacttacactctttaagccattccagtcatgatgaggtggaatgtatcagtataccaattaatatttttgaaagagttcttttaggttaatttaagtacagcaatttctcatgtaatgtttagggagtttattctaacctaggcaaacggcatgctatcacaagaaaggtttaaagctttgataaaatgggggagatttaatcagtttttttaatgcctgctataaaaatttgaaatattagaatggccgaccatggcagtgaccaggcctcactacaggcctggttggattctggtctttaatgcatgctagtgttgatgttttttggtcaagaacggtttaaacaggaaggattgtgcagcaggctttaatttaatgtagattcatactgctctgttaaagctgcattgaaatgttaaaatggcttacacttgcagactttgcaaatcttaagactaacaaatccttgaaatcacacagcttgcaaatacgtactaaactgcacaaggtgtgtgttctatatgtgcagttttagcgtattttagttgcataggtttccatggtatttatagtctcttgtgctaaatttggccaaagatgattgtccaccactaaaaatgcctctcccacttggaattctgtactgattttgtggccagatgcaatgatctttaaaaacaaatcttttcaatggcataagaagttgacaaaaatttcttaaagtgcaatagattttcaagttattgtgccttgttctaaaattttaagtagggcacttgacagtattgaggtcatttgttaaggtgctatttcaattagtgtaggtttagactcttgtacatttctcccataactttttacaaagtattttgttgcacattcagagaattttatatatatatgtcttgtgtgggtgtcctcgaccttccaatcttatttcgtctcttggagattgttgaatgcagccagtgaagaagtagattcctaaattttattggggaccatggaatggtagttgagaagaaaactatttgcacacaacagattttagatactttttgctgctagttgtgtaatatttattgaacattttgacaaatatttatttttgtaagcctaaaaatgattctttgaaagtttaaagaaacttgaccaaaagacagtacaaaaaacactggcacttgaatgttgaatgtcaccgtatgtgaaataatatattttggggtagtgtgagcttttaatgttaagtctgttaaacttgagtcaaattaagcagacccggcattggcaatgtagctgtaattttctgacaaaatttaagacaaaattgtcaacttgaaactaaaacatgccaaggttttgatatacttgtcttaagatattaatgaaacaattttgaacactgataggaaggtccacatccacaaagtttctcttgagttttgttatgtgttttgctgtgtttgattttcagtgattgtctggtatatttacagtcctcaaacatggttatttctgtcagtgacttaacattcggttttaccagccagcagtattcttcagtaaataaagaatggaattgctgaatgtaatcattgaacctcgagtcactgtaaaagttcagtaattgcttattgtattagttttagatgctggcaccgcatgtgctctgtttattctgattttactaaaataaaaagttcaaaagtcaaaaaaaaaa

SEQ ID NO: 6 - protein, 144 aa, Homo sapiens
MPKNKGKGGKNRRRGKNENESEKRELVFKEDGQEYAQVIKMLGNGRLEALCFDGVKRLCHIRGKLRKKVWINTSDIILVGLRDYQDNKADVILKYNADEARSLKAYGELPEHAKINETDTFGPGDDDEIQFDDIGDDDEDIDDI

SEQ ID NO: 7 - RNA, 1384 nt, Homo sapiens
  source 1..1384: mol_type = mRNA
gcagtttatgagagagctctgtagccagcctcttctgcgcacccacctgctgcatcttagttcagtcggctcttagagtagtaaccgccagaaaggagtcggaagaggtctcacgaggctgtcatcaccgccatgcccaagaataaaggtaaaggaggtaaaaacaggcgcaggggtaaaaatgagaatgaatctgaaaaaagagagttggtgtttaaagaggatggacaagagtatgctcaggtaatcaaaatgttgggaaatggacgattggaagcattgtgttttgatggtgtaaagaggttatgccatatcagagggaaattgagaaaaaaggtttggataaatacatcagacattatattggttggtctacgggactatcaggataacaaagctgatgtaattttaaagtacaatgcagatgaagctagaagcctgaaggcatatggcgggcttccagaacatgctaaaatcaatgaaacagacacatttggtcctggagatgatgatgaaatccagtttgacgatattggagatgatgatgaagacattgatgatatctaaattgaaccaagtgtttttacatgacaagttctctgaggatggttctacagttgggattttggccatcatcaaccaagaagagaaattcatttagtgtgtagtttctgaaagcaaactgatttattttcattgttttaaagtatttatttctttaaaagctgaggacattgaattaccttaatttaaatgttaatactttattgttttgatgtaatggaacttaaggataaaagaccataatatttgctgttaaaataaataaacgagtgcctttcctactgtgataacgtcaagtaattggatattttgaatacatttctgcctgataatcatgctgagttctaataagccctacttccacctaatctgtttacagtcttttggtatgtttcagttacttagatggtctcataaggtttctgatacaatttgaagacagaaatctgcatttagaatcagaaaacatggacatatttttcatatttatctagtcatatgtaattttatgctaacattgatagtttataaatccttttcatcctttgtgcctcggttattaaggaaaaaaaaatgtccaacatacagtttttaaagtgtggcagttttgagtagtaacttagaatgtataagattaagagttaaagaaaccgaacaataagtggcaaccaattatcttaacattggaaatactggggtgccattttgttttcaaaagttattcattgtaatccactgttttggctttcatgaacaagtaaattacagtgtataaatgaaaagcaatttcataataaattctataaactgaaaaaaaaaa

SEQ ID NO: 8 - protein, 1347 aa, Homo sapiens [sequence omitted]

SEQ ID NO: 9 - RNA, 4335 nt, Homo sapiens
  source 1..4335: mol_type = mRNA
gctcatcgtttgttgtttagataatatcatgaactgataaatgcagttgccacgttgattccctagggcctggcttaccgactgaggtcataagatattatgccttctctttagacttggtcagtggagaggaaatgggcaaagaaccagcctatggaggtgacaaggccttagggccaaaagtcttgagggtgaaggtttagggcctgcgcagcttccctgccatgccccgcaaggtctcgcattcgcaaggcttgtgacagtgggagcctcattacggactctcctaaagtccatggtgtcctcttttcgcatttgcgccccgtgggtgatgcccgatgccgcccttcccatcgctctcttccccttcaagcgtatcgcaactgcaaaaacacccagcacagacactccattttctatcttaatgcatttaactagcacaacctacaggttgttccatcccagagactacccttttctccatagacgtgaccatcaaccaaccagcggtcagaatcagtcagcctctgtcatgttcctaggtccttggcgaactggctgggcggggtcccagcagcctaggagtacagtggagcaatgcctgacgtaagtcaacaaagatcacgtgagacgaatcagtcgcctagattggctacaactaagtggttgggagcggggaggtcgcggcggctgcgtggggttcgcccgtgacacaattacaactttgtgctggtgctggcaaagtttgtgattttaagaaattctgctgtgctctccagcactgcgagcttctgccttccctgtagtttcccagatgtgatccaggtagccgagttccgctgcccgtgcttcggtagcttaagtctttgcctcagcttttttccttgcagccgctgaggaggcgataaaattggcgtcacagtctcaagcagcgattgaaggcgtcttttcaactactcgattaaggttgggtatcgtcgtgggacttggaaatttgttgtttccatgaaatcctgcgcagtgtcgctcactaccgccgctgttgccttcggtgatgaggcaaagaaaatggcggaaggaaaagcgagccgcgagagtgaagaggagtctgttagcctgacagtcgaggaaagggaggcgcttggtggcatggacagccgtctcttcgggttcgtgaggcttcatgaagatggcgccagaacgaagaccctactaggcaaggctgttcgctgctacgaatctttaatcttaaaagctgaaggaaaagtggagtctgacttcttttgccaattaggtcacttcaacctcttgttggaagattattcaaaagcattatctgcatatcagagatattacagtttacaggctgactactggaagaatgctgcgtttttatatggccttggtttggtctacttctactacaatgcatttcattgggcaattaaagcatttcaagatgtcctttatgttgaccccagcttttgtcgagccaaggaaattcatttacgacttgggctcatgttcaaagtgaacacagactacaagtctagtttaaagcattttcagttagccttgattgactgtaatccatgtactttgtccaatgctgaaattcaatttcatattgcccatttgtatgaaacccagaggaagtatcattctgcaaaggaggcatatgaacaacttttgcagacagaaaaccttcctgcacaagtaaaagcaactgtattgcaacagttaggttggatgcatcataatatggatctagtaggagacaaagccacaaaggaaagctatgctattcagtatctccaaaagtctttggaggcagatcctaattctggccaatcgtggtattttcttggaaggtgttattcaagtattgggaaagttcaggatgcctttatatcttacaggcaatctattgataaatcagaagcaagtgcagatacatggtgttcaataggtgtgttgtatcagcagcaaaatcagcctatggatgctttacaggcatatatttgtgctgtacaattggaccatgggcatgccgcagcctggatggacctaggtactctctatgaatcctgcaatcaacctcaagatgccattaaatgctacctaaatgcagctagaagcaaacgttgtagtaatacctctacgcttgctgcaagaattaaatttctacagaatggttctgataactggaatggtggccagagtctttcacatcatccagtacagcaagtttattcgttgtgtttgacaccacagaaattacagcacttggaacaactgcgagcaaatagagataatttaaatccagcacagaagcatcagctggaacagttagaaagtcagtttgtcttaatgcagcaaatgagacacaaagaagttgctcaggtacgaactactggaattcataacggggccataactgattcatcactgcctacaaactctgtctctaatcgacaaccacatggtgctctgaccagagtatctagcgtctctcagcctggagttcgccctgcttgtgttgaaaaacttttgtccagtggagctttttctgcaggctgtattccttgtggcacatcaaaaattctaggaagtacagacactatcttgctaggcagtaattgtatagcaggaagtgaaagtaatggaaatgtgccttacctgcagcaaaatacacacactctacctcataatcatacagacctgaacagcagcacagaagagccatggagaaaacagctatctaactccgctcaggggcttcataaaagtcagagttcatgtttgtcaggacctaatgaagaacaacctctgttttccactgggtcagcccagtatcaccaggcaactagcactggtattaagaaggcgaatgaacatctcactctgcctagtaattcagtaccacagggggatgctgacagtcacctctcctgtcatactgctacctcaggtggacaacaaggcattatgtttaccaaagagagcaagccttcaaaaaatagatccttggtgcctgaaacaagcaggcatactggagacacatctaatggctgtgctgatgtcaagggactttctaatcatgttcatcagttgatagcagatgctgtttccagtcctaaccatggagattcaccaaatttattaattgcagacaatcctcagctctctgctttgttgattggaaaagccaatggcaatgtgggtactggaacctgcgacaaagtgaataatattcacccagctgttcatacaaagactgatcattctgttgcctcttcaccctcttcagccatttccacagcaacaccttctcctaaatccactgagcagagaagcataaacagtgttaccagccttaacagtcctcacagtggattacacacagtcaatggagaggggctggggaagtcacagagctctacaaaagtagacctgcctttagctagccacagatctacttctcagatcttaccatcaatgtcagtgtctatatgccccagttcaacagaagttctgaaagcatgcaggaatccaggtaaaaatggcttgtctaatagctgcattttgttagataaatgtccacctccaagaccaccaacttcaccatacccacccttgccaaaggacaagttgaatccacccacacctagtatttacttggaaaataaacgtgatgctttctttcctccattacatcaattttgtacaaatccaaaaaaccctgttacagtaatacgtggccttgctggagctcttaaattagatcttggacttttctctaccaaaactttggtagaagctaacaatgaacatatggtagaagtgaggacacagttgctgcaaccagcagatgaaaactgggatcccactggaacaaagaaaatctggcgttgtgaaagcaatagatctcatactacaattgccaaatacgcacaataccaggcttcctccttccaggaatcattgagagctggaatgcaatggtgtgatctcagctcactgcagcctccgcctcctgggttcaagcgattctcccacctcagcctcccgaatagctggaattacaggcacctgccatcatgcccaactaatttttgtatttttgtagagacagggtttcaccatgttggccaggcttgtcttgaactcctgacctcaggtggtctgcttgcctcagcatcccaaagtgctgggattacaggtgtgagccaccatgcccggtaaacttttaaaaatgtaagcaaaattacagtatgtaaaacacacattgctaatggagaaataaagttcctacttttacatctaaaaaaaaaa

SEQ ID NO: 10 - protein, 801 aa, Homo sapiens
MDEDEFELQPQEPNSFFDGIGADATHMDGDQIVVEIQEAVFVSNIVDSDITVHNFVPDDPDSVVIQDVVEDVVIEEDVQCSDILEEADVSENVIIPEQVLDSDVTEEVSLPHCTVPDDVLASDITSTSMSMPEHVLTSESMHVCDIGHVEHMVHDSVVEAEIITDPLTSDIVSEEVLVADCAPEAVIDASGISVDQQDNDKASCEDYLMISLDDAGKIEHDGSTGVTIDAESEMDPCKVDSTCPEVIKVYIFKADPGEDDLGGTVDIVESEPENDHGVELLDQNSSIRVPREKMVYMTVNDSQQEDEDLNVAEIADEVYMEVIVGEEDAAVAAAAAAVHEQQIDEDEMKTFVPIAWAAAYGNNSDGIENRNGTASALLHIDESAGLGRLAKQKPKKKRRPDSRQYQTAIIIGPDGHPLTVYPCMICGKKFKSRGFLKRHMKNHPEHLAKKKYHCTDCDYTTNKKISLHNHLESHKLTSKAEKAIECDECGKHFSHAGALFTHKMVHKEKGANKMHKCKFCEYETAEQGLLNRHLLAVHSKNFPHICVECGKGFRHPSELRKHMRIHTGEKPYQCQYCEYRSADSSNLKTHIKTKHSKEMPFKCDICLLTFSDTKEVQQHTLVHQESKTHQCLHCDHKSSNSSDLKRHVISVHTKDYPHKCEMCEKGFHRPSELKKHVAVHKGKKMHQCRHCDFKIADPFVLSRHILSVHTKDLPFRCKRCRKGFRQQNELKKHMKTHSGRKVYQCEYCEYSTTDASGFKRHVISIHTKDYPHRCEYCKKGFRRPSEKNQHIMRHHKEVGLP

SEQ ID NO: 11 - RNA, 2659 nt, Homo sapiens
  source 1..2659: mol_type = mRNA
atggatgaagatgaatttgaattgcagccacaagagccaaactcattttttgatggaataggagctgatgctacacacatggatggtgatcagattgttgtggaaatacaagaagcagtttttgtttctaatattgtggattctgacataactgtgcataactttgttcctgatgacccagactcagttgtaatccaagatgttgttgaagatgttgtcatagaggaggatgttcagtgctcagatatcttagaagaggcagatgtatctgaaaatgtcatcattcctgagcaagtgctggactcagatgtaactgaagaagtttctttaccacactgcacagtcccagatgatgttttagcttctgacattacttcaacctcaatgtctatgccagaacatgttttaacgagtgaatccatgcatgtgtgtgacattggacatgttgaacatatggtgcatgatagtgtagtggaagcagaaatcattactgatcctctgacgagtgacatagtttcagaagaagtattggtagcagactgtgcccctgaagcagtcatagatgccagcgggatctcagtggaccagcaagataatgacaaagccagctgtgaggactacctaatgatttcgttggatgatgctggcaaaatagaacatgatggttccactggagtgaccatcgatgcagaatcagaaatggatccttgtaaagtggatagcacttgtcctgaagtcatcaaggtgtacatttttaaagctgaccctggagaagatgacttaggtggaactgtagacattgtggagagtgaacctgaaaatgatcatggagttgaactacttgatcagaacagcagtattcgtgttcccagggaaaagatggtttatatgactgtcaatgactctcaacaagaagatgaagatttaaatgttgctgaaattgctgatgaagtttatatggaagtgatcgtaggagaggaggatgctgctgttgcagcagcagcagctgctgtgcatgagcagcaaattgatgaggatgaaatgaaaaccttcgtaccaattgcatgggcagcagcttatggtaataattctgatggaattgaaaaccggaatggcactgcaagtgccctcttgcacatagatgagtctgctggccttggcagactggctaaacagaaaccaaagaaaaagagaagacctgattccaggcagtaccaaacagcaataattattggccctgatggtcatcctttgactgtctatccttgcatgatttgtgggaagaagtttaagtcgaggggttttttgaaaagacacatgaaaaaccatcctgaacaccttgccaagaagaagtaccactgtactgactgtgattacactaccaataagaagataagtttacataaccacctggagagccacaagctgaccagcaaggcagagaaggccattgaatgtgatgagtgtgggaagcatttttctcatgcaggggctttgtttactcacaaaatggtgcataaggaaaaaggggccaacaaaatgcacaagtgtaaattctgtgaatatgagacagctgaacaggggttattgaatcgccacctcttggcagtccacagcaagaactttcctcatatttgtgtggagtgtggtaaaggtttccgatacccgtcggaactgagaaagcacatgcgaatccataccggcgagaagccataccaatgccagtactgtgaatataggtctgcagactcttctaacttgaaaacacatataaaaacaaagcatagtaaagagatgccattcaagtgtgacatttgtcttctgactttctcagataccaaagaagtgcagcaacatactcttgtccaccaagaaagcaaaacacatcagtgtttgcattgcgaccacaagagttcaaactcaagtgatttgaaacgacatgtaatttcagttcatacgaaagactatcctcataagtgtgagatgtgcgagaaaggctttcacaggccttcagaacttaagaaacatgtggctgtccacaaaggtaaaaaaatgcaccaatgtagacattgtgactttaagattgcagacccatttgttctaagtcgccatattctctcagttcacacaaaggatcttccatttaggtgtaagagatgtagaaagggatttaggcaacaaaatgagcttaaaaagcatatgaagacacacagtggcaggaaagtatatcagtgtgagtactgtgagtatagcactacagatgcctcaggctttaaacggcacgttatttccattcatacaaaagactatcctcatcggtgtgagtactgcaagaaaggcttccgaagaccttcagaaaagaaccagcacataatgagacaccataaagaagttggtctgccctaacagtgtgtctacaagcttgtaaagatgttggccttgaagcagaaaattcattttttaaagccagtcttgttcacatccattactatacattgaattatgctgtgtaaaaatagaattattgcttctagtccacttttctttacattttattcaatacgctgtcctgaatcctattcagtttctttaatagatgagtaaaaatagcaacaagcaagttgcttataataaaataatttgtgattctcccgaattc

SEQ ID NO: 12 - protein, 1539 aa, Homo sapiens
MEPGCDEFLPPPECPVFEPSWAEFQDPLGYIAKIRPIAEKSGICKIRPPADWQPPFAVEVDNFRFTPRVQRLNELEAQTRVKLNYLDQIAKFWEIQGSSLKIPNVERKILDLYSLSKIVIEEGGYEAICKDRRWARVAQRLHYPPGKNIGSLLRSHYERIIYPYEMFQSGANHVQCNTHPFDNEVKDKEYKPHSIPLRQSVQPSKFSSYSRRAKRLQPDPEPTEEDIEKHPELKKLQIYGPGPKMMGLGLMAKDKDKTVHKKVTCPPTVTVKDEQSGGGNVSSTLLKQHLSLEPCTKTTMQLRKNHSSAQFIDSYICQVCSRGDEDDKLLFCDGCDDNYHIFCLLPPLPEIPRGIWRCPKCILAECKQPPEAFGFEQATQEYSLQSFGEMADSFKSDYFNMPVHMVPTELVEKEFWRLVSSIEEDVTVEYGADIHSKEFGSGFPVSNSKQNLSPEEKEYATSGWNLNVMPVLDQSVLCHINADISGMKVPWLYVGMVFSAFCWHIEDHWSYSINYLHWGEPKTWYGVPSLAAEHLEEVMKMLTPELFDSQPDLLHQLVTLMNPNTLMSHGVPVVRTNQCAGEFVITFPRAYHSGFNQGYNFAEAVNFCTADWLPAGRQCIEHYRRLRRYCVFSHEELICKMAAFPETLDLNLAVAVHKEMFIMVQEERRLRKALLEKGVTEAEREAFELLPDDERQCIKCKTTCFLSALACYDCPDGLVCLSHINDLCKCSSSRQYLRYRYTLDELPTMLHKLKIRAESFDTWANKVRVALEVEDGRKRSFEELRALESEARERRFPNSELLQRLKNCLSEVEACIAQVLGLVSGQVARMDTPQLTLTELRVLLEQMGSLPCAMHQIGDVKDVLEQVEAYQAEAREALATLPSSPGLLRSLLERGQQLGVEVPEAHQLQQQVEQAQWLDEVKQALAPSAHRGSLVIMQGLLVMGAKIASSPSVDKARAELQELLTIAERWEEKAHFCLEARQKHPPATLEAIIRETENIPVHLPNIQALKEALTKAQAWIADVDEIQNGDHYPCLDDLEGLVAVGRDLPVGLEELRQLELQVLTAHSWREKASKTFLKKNSCYTLLEVLCPCADAGSDSTKRSRWMEKALGLYQCDTELLGLSAQDLRDPGSVIVAFKEGEQKEKEGILQLRRTNSAKPSPLAPSLMASSPTSICVCGQVPAGVGVLQCDLCQDWFHGQCVSVPHLLTSPKPSLTSSPLLAWWEWDTKFLCPLCMRSRRPRLETILALLVALQRLPVRLPEGEALQCLTERAIGWQDRARKALASEDVTALLRQLAELRQQLQAKPRPEEASVYTSATACDPIREGSGNNISKVQGLLENGDSVTSPENMAPGKGSDLELLSSLLPQLTGPVLELPEAIRAPLEELMMEGDLLEVTLDENHSIWQLLQAGQPPDLDRIRTLLELEKFEHQGSRTRSRALERRRRRQKVDQGRNVENLVQQELQSKRARSSGIMSQVGREEEHYQEKADRENMFLTPSTDHSPFLKGNQNSLQHKDSGSSAACPSLMPLLQLSYSDEQQL

SEQ ID NO: 13 - RNA, 5476 nt, Homo sapiens
  source 1..5476: mol_type = mRNA
ggacggccatactatttttatcttgctttttcgttctgtcgcagtactgtttaatatgagtccagcgacggctctgtgactgttttcctctggtaaaatcgctcttgcgtcctcagcgtttatctcaggtgcggaaggtctcacaggtttggaaatagcgccggaaaaatcgatccgcggagtgagacggctcgtaccacactgcagggcccggaggtcaagatggtggctgtaaaactaggatccctgacgattgcttagcattaaggcccgacatggaaccggggtgtgacgagttcctgccgccaccggagtgcccggtttttgagcctagctgggctgaattccaagacccgcttggctacattgcgaaaataaggcccatagcagagaagtctggcatctgcaaaatccgcccacccgcggattggcagcctccttttgcagtagaagttgacaatttcagatttactcctcgcgtccaaaggctaaatgaactggaggcccaaactagagtgaaattgaactatttggatcagattgcaaaattctgggaaattcaaggctcctctttaaagattcccaatgtggagcggaagatcttggacctctacagccttagtaagattgtgattgaggaaggtggctatgaagccatctgcaaggatcgtcggtgggctcgagttgcccagcgtctccactacccaccaggcaaaaacattggctccctgctacgatcacattacgaacgcattatttacccctatgaaatgtttcagtctggagccaaccatgtgcaatgtaacacacacccgtttgacaatgaggtaaaagataaggaatacaagccccacagcatcccccttagacagtctgtgcagccttcaaagttcagcagctacagtcgacgggcaaaaaggctacagcctgatccagagcctacagaggaggacattgagaagcatccagagctaaagaagttacagatatatgggccaggtcccaaaatgatgggcttgggccttatggctaaggataaggataagactgtgcataagaaagtcacatgccccccaactgttacggtgaaggatgagcaaagtggaggtgggaacgtgtcatcaacattgctcaagcagcacttgagcctagagccctgcactaagacaaccatgcaacttcgaaagaatcacagcagtgcccagtttattgactcatatatttgccaagtatgctcccgtggggatgaagataataagcttcttttctgtgatggctgtgatgacaattaccacatcttctgcttgttaccaccccttcctgaaatccccagaggcatctggaggtgcccaaaatgtatcttggcggagtgtaaacagcctcctgaagcttttggatttgaacaggctacccaggagtacagtttgcagagttttggtgaaatggctgattccttcaagtccgactacttcaacatgcctgtacatatggtgcctacagaacttgtagagaaggaattctggaggctggtgagcagcattgaggaagacgtgacagttgaatatggagctgatattcattccaaagaatttggcagtggctttcctgtcagcaatagcaaacaaaacttatctcctgaggagaaggagtatgcgaccagtggttggaacctgaatgtgatgccagtgctagatcagtctgttctctgtcacatcaatgcagacatctcaggcatgaaggtgccctggctgtacgtgggcatggttttctcagcattttgttggcatattgaggatcactggagttactctattaactatctgcattggggtgagccgaagacctggtatggtgtaccctccctggcagcagagcatttggaggaggtgatgaagatgctgacacctgagctgtttgatagccagcctgatctcctacaccagcttgtcactctcatgaatcccaacactttgatgtcccatggtgtgccagttgtccgcacaaaccagtgtgcaggggagtttgtcatcacttttcctcgtgcttaccacagtggttttaaccaaggctacaattttgctgaagctgtcaacttttgtactgctgactggctacctgctggacgccagtgcattgaacactaccgccggctccggcgctattgtgtcttctcccacgaggagctcatctgcaagatggctgccttcccagagacgttggatctcaatctagcagtagctgtgcacaaggagatgttcattatggttcaggaggagcgacgtctacgaaaggcccttttggagaagggcgtcacggaggctgagcgagaggcttttgagctgctcccagatgatgaacgccagtgcatcaagtgcaagaccacgtgcttcttgtcagccctggcctgctacgactgcccagatggccttgtatgcctttcccacatcaatgacctctgcaagtgctctagtagccgacagtacctccggtatcggtacaccttggatgagctccccaccatgctgcataaactgaagattcgggctgagtcttttgacacctgggccaacaaagtgcgagtggccttggaggtggaggatggccgtaaacgcagctttgaagagctaagggcactggagtctgaggctcgtgagaggaggtttcctaatagtgagctgcttcagcgactgaagaactgcctgagtgaggtggaggcttgtattgctcaagtcctggggctggtcagtggtcaggtggccaggatggacactccacagctgactttgactgaactccgggtccttcttgagcagatgggcagcctgccctgcgccatgcatcagattggggatgtcaaggatgtcctggaacaggtggaggcctatcaagctgaggctcgtgaggctctggccacactgccctctagtccagggctattgcggtccctgttggagagggggcagcagctgggtgtagaggtgcctgaagcccatcagcttcagcagcaggtggagcaggcgcaatggctagatgaagtgaagcaggccctggccccttctgctcacaggggctctctggtcatcatgcaggggcttttggttatgggtgccaagatagcctccagcccttctgtggacaaggcccgggctgagctgcaagaactactgaccattgcagagcgctgggaagaaaaggctcatttctgcctggaggccaggcagaagcatccaccagccacattggaagccataattcgtgagacagaaaacatccctgttcacctgcctaacatccaggctctcaaagaagctctgactaaggcacaagcttggattgctgatgtggatgagatccaaaatggtgaccactacccctgtctagatgacttggagggcctggtggctgtgggccgggacctgcctgtggggctggaagagctgagacagctagagctgcaggtattgacagcacattcctggagagagaaggcctccaagacctttctcaagaagaattcttgctacacactgcttgaggtgctttgcccgtgtgcagacgctggctcagacagcaccaagcgtagccggtggatggagaaggcgctggggttgtaccagtgtgacacagagctgctggggctgtctgcacaggacctcagagacccaggctctgtgattgtggccttcaaggaaggggaacagaaggagaaggagggtatcctgcagctgcgtcgcaccaactcagccaagcccagtccactggcaccatccctcatggcctcttctccaacttctatctgtgtgtgtgggcaggtgccagctggggtgggacttctgcagtgtgacctgtgtcaggactggttccatgggcagtgtgtgtcagtgccccatctcctcacctctccaaagcccagtctcacttcatctccactgctagcctggtgggaatgggacacaaaattcctgtgtccactgtgtatgcgctcacgacggccacgcctagagacaatcctagccttgctggttgccctgcagaggctgcccgtgcggctgcctgagggtgaggcccttcagtgtctcacagagagggccattggctggcaagaccgtgccagaaaggctctggcctttgaagatgtgactgctctgttgcgacagctggctgagcttcgccaacagctacaggccaaacccagaccagaggaggcctcagtctacacttcagccactgcctgtgaccctatcagagaaggcagtggcaacaatatttctaaggtccaagggctgctggagaatggagacagtgtgaccagtcctgagaacatggctccaggaaagggctctgacctggagctactgtcctcgctgttgccgcagttgactggccctgtgttggagctgcctgaggcaatccgggctcccctggaggagctcatgatggaagggggcctgcttgaggtgaccctggatgagaaccacagcatctggcagctgctgcaggctggacagcctccagacctggacagaattcgcacacttctggagctggaaaaatttgaacatcaagggagtcggacaaggagccgggctctggagaggcgacggcggcggcagaaggtggatcagggtagaaacgttgagaatcttgttcaacaggagcttcagtcaaaaagggctcggagctcagggattatgtctcaggtgggccgagaagaagaacattatcaggagaaagcagaccgtgaaaatatgttcctgacaccttccacagaccacagccctttcttgaaaggaaaccaaaatagcttacaacacaaggattcaggctcttcagctgcttgtccttctttaatgcctttgctacaactctcctactctgatgagcaacagttgtgacagtggcaccaaaggtcatttgtggttgtttttgtttgtttgtttcttaaatcctactatctcctggcctggacctcagaaggagctttttgcctatctataatttttcactgccaatttttgatatcctctctcctagagttactgttaaaaggttggttcgtaaagtccacaccccgatgctcagaagtgtcttgccagcaacattcctgctagcatacaggagtgatttcctaaaccagtttcattctagtctgaatagggacaaacaaatcttgaggaagcccaagtgcgtacctttatttttgcccccaccaccctctttctgtacttcaatttttgtttgttttttgtttttttgtccctgtcataaaatattttggtgcttcaaaacttgtaccttcattgtacatccttttcttttctccccttgggtcttattataaaagaagacaatgtacgttgtaattaccaaaaagaatagggaaaaacaagaatttcatgactctacctgtggtctatctttaatttcatttcttttgttaaaaataaaacaatgagtatgtttgggaaaaaaaaaa

SEQ ID NO: 14 - protein, 2555 aa, Homo sapiens
MTAITHGSPVGGNDSQGQVLDGQSQHLFQQNQTSSPDSSNENSVATPPPEEQGQGDAPPQHEDEEPAFPHTELANLDDMINRPRWVVPVLPKGELEVLLEAAIDLSVKGLDVKSEACQRFFRDGLTISFTKILMDEAVSGWKFEIHRCIINNTHRLVELCVAKLSQDWFPLLELLAMALNPHCKFHIYNGTRPCELISSNAQLPEDELFARSSDPRSPKGWLVDLINKFGTLNGFQILHDRFFNGSALNIQIIAALIKPFGQCYEFLSQHTLKKYFIPVIEIVPHLLENLTDEELKKEAKNEAKNDALSMIIKSLKNLASRISGQDETIKNLEIFRLKMILRLLQISSFNGKMNALNEINKVISSVSYYTHRHSNPEEEEWLTAERMAEWIQQNNILSIVLQDSLHQPQYVEKLEKILRFVIKEKALTLQDLDNIWAAQAGKHEAIVKNVHDLLAKLAWDFSPGQLDHLFDCFKASWTNASKKQREKLLELIRRLAEDDKDGVMAHKVLNLLWNLAQSDDVPVDIMDLALSAHIKILDYSCSQDRDAQKIQWIDHFIEELRTNDKWVIPALKQIREICSLFGEASQNLSQTQRSPHIFYRHDLINQLQQNHALVTLVAENLATYMNSIRLYAGDHEDYDPQTVRLGSRYSHVQEVQERLNFLRFLLKDGQLWLCAPQAKQIWKCLAENAVYLCDREACFKWYSKLMGDEPDLDPDINKDFFESNVLQLDPSLLTENGMKCFERFFKAVNCRERKLIAKRRSYMMDDLELIGLDYLWRVVIQSSDEIANRAIDLLKEIYTNLGPRLKANQVVIHEDFIQSCFDRLKASYDTLCVFDGDKNSINCARQEAIRMVRVLTVIKEYINECDSDYHKERMILPMSRAFRGKHLSLIVRFPNQGRQVDELDIWSHTNDTIGSVRRCIVNRIKANVAHKKIELFVGGELIDSEDDRKLIGQLNLKDKSLITAKLTQINFNMPSSPDSSSDSSTASPGNHRNHYNDGPNLEVESCLPGVIMSVHPRYISFLWQVADLGSNLNMPPLRDGARVLMKLMPPDRTAVEKLRAVCLDHAKLGEGKLSPPLDSLFFGPSASQVLYLTEVVYALLMPAGVPLTDGSSDFQVHFLKSGGLPLVLSMLIRNNFLPNTDMETRRGAYLNALKIAKLLLTAIGYGHVRAVAEACQPVVDGTDPITQINQVTHDQAVVLQSALQSIPNPSSECVLRNESILLAQEISNEASRYMPDICVIRAIQKIIWASACGALGLVFSPNEEITKIYQMTTNGSNKLEVEDEQVCCEALEVMTLCFALLPTALDALSKEKAWQTFIIDLLLHCPSKTVRQLAQEQFFLMCTRCCMGHRPLLFFITLLFTILGSTAREKGKYSGDYFTLLRHLLNYAYNGNINIPNAEVLLVSEIDWLKRIRDNVKNTGETGVEEPILEGHLGVTKELLAFQTSEKKYHFGCEKGGANLIKELIDDFIFPASKVYLQYLRSGELPAEQAIPVCSSPVTINAGFELLVALAIGCVRNLKQIVDCLTEMYYMGTAITTCEALTEWEYLPPVGPRPPKGFVGLKNAGATCYMNSVIQQLYMIPSIRNSILAIEGTGSDLHDDMFGDEKQDSESNVDPRDDVFGYPHQFEDKPALSKTEDRKEYNIGVLRHLQVIFGHLAASQLQYYVPRGFWKQFRLWGEPVNLREQHDALEFFNSLVDSLDEALKALGHPAILSKVLGGSFADQKICQGCPHRYECEESFTTLNVDIRNHQNLLDSLEQYIKGDLLEGANAYHCEKCDKKVDTVKRLLIKKLPRVLAIQLKRFDYDWERECAIKFNDYFEFPRELDMGPYTVAGVANLERDNVNSENELIEQKEQSDNETAGGTKYRLVGVLVHSGQASGGHYYSYIIQRNGKDDQTDHWYKFDDGDVTECKMDDDEEMKNQCFGGEYMGEVFDHMMKRMSYRRQKRWWNAYILFYEQMDMIDEDDEMIRYISELTIARPHQIIMSPAIERSVRKQNVKFMHNRLQYSLEYFQFVKKLLTCNGVYLNPAPGQDYLLPEAEEITMISIQLAARFLFTTGFHTKKIVRGPASDWYDALCVLLRHSKNVRFWFTHNVLFNVSNRFSEYLLECPSAEVRGAFAKLIVFIAHFSLQDGSCPSPFASPGPSSQACDNLSLSDHLLRATLNLLRREVSEHGHHLQQYFNLFVMYANLGVAEKTQLLKLNVPATFMLVSLDEGPGPPIKYQYAELGKLYSVVSQLIRCCNVSSTMQSSINGNPPLPNPFGDLNLSQPIMPIQQNVLDILFVRTSYVKKIIEDCSNSEDTIKLLRFCSWENPQFSSTVLSELLWQVAYSYTYELRPYLDLLFQILLIEDSWQTHRIHNALKGIPDDRDGLFDTIQRSKNHYQKRAYQCIKCMVALFSSCPVAYQILQGNGDLKRKWTWAVEWLGDELERRPYTGNPQYSYNNWSPPVQSNETANGYFLERSHSARMTLAKACELCPEEEPDDQDAPDEHEPSPSEDAPLYPHSPASQYQQNNHVHGQPYTGPAAHHLNNPQKTGQRTQENYEGNEEVSSPQMKDQ

SEQ ID NO: 15 - RNA, 9372 nt, Homo sapiens
  source 1..9372: mol_type = mRNA
tgaataattgaactttgtttatttctccatatttttgcagtggtaattccattataaaacctaatgaaacaatgtttttatagatggtgtggaaagacttttctgggctcagaggtgaaactgacccttgtgtatcagcagcatttctgactgactgagagagtgtagtgattaacagagttgtgatgttagttaagaaacttagatttgccattgtagcttttctaccaattagcagattgtttaactcactgaaattgtaaagtggtagacgtggacttagtcattactgggcagcttatgaattgtattcatttactcatgatgtaaaaatggttagtctccacttttaaggctctagttctagtggctaaataggtacttatttatacagtatgataactgctgtattaaaatacatgtctcaaatgtggaatagtagaagaggtgaagaaaatcatagtttgaggtagaatactgtttgctggtcttaaaaactgtggtattttggtgattccataaattaggtcagatacttccactggagggaaacagtttaaaggatatatgtgatactattaatagaatgaggaagacacaccagatatttaggagggaattagcgagcttgaaactaagagctggtttgaatgagactgggtcataagtgatttcaagtaccagattaaggcactgagattttatttttaagcactgaagtcagattttttccttttaaaagaaaggattcatgatgaaatctgctttttgttttgcagagagcttggagataattctggtggctgtgtggagtatgtgttggaggtattaaattttcacagtatatataaggcagcaattgataggcctttcacagattcttctgataactacataaagagacaaaaaaaagaaaaaagagcaaagatctgtgctgtgtcaagtatgacagccatcactcatggctctccagtaggagggaacgacagccagggccaggttcttgatggccagtctcagcatctcttccaacagaaccagacttcatcacctgattcttccaatgagaattccgtagcaactcctcctccagaggaacaagggcaaggtgatgccccaccacagcatgaagatgaagagcctgcatttccacatactgagctggcaaacctggatgacatgatcaacaggcctcgatgggtggttcctgttttgccaaaaggggaattagaagtgcttttagaagctgctattgatcttagtgtaaaaggccttgatgttaaaagtgaagcatgccaacgtttttttcgagatggactaacaatatctttcactaaaattcttatggatgaggctgtgagtggctggaagtttgaaattcatagatgtattattaacaatactcatcgcctagtggagctttgtgtggccaagttgtcccaagattggtttccacttctagaacttctcgccatggccttaaatcctcactgcaagtttcatatctacaatggtacacgtccgtgtgaattaatttcctcaaatgctcagttgcctgaagatgaattatttgctcgttcttcagatcctcgatcaccaaaaggttggctagtggatctcatcaataaatttggcacattaaatgggttccagattttgcatgatcgtttttttaatggatcagcattaaatattcaaataattgcagctcttattaaaccatttggacaatgctatgagtttctcagtcaacatacactgaaaaagtacttcattccagttatagaaatggttccacatttattggaaaacttaactgatgaagaactgaaaaaggaggcaaagaatgaagccaaaaatgatgccctttcaatgattattaaatctttgaagaacttagcttcaagaatttcaggacaagatgagactataaaaaatttggaaatttttaggttaaagatgatactcagattgttgcaaatttcctcttttaatggaaagatgaatgcactgaatgaaataaataaggttatatctagtgtatcatattatactcatcggcatagtaatcctgaggaggaagaatggctgacagctgagcgaatggcagaatggatacagcaaaataatatcttatccatagtcttgcaagacagtcttcatcaaccacaatatgtagaaaagctagagaaaattcttcgttttgtgattaaagaaaaggctcttacattacaggaccttgataatatctgggcagcacaggcaggaaaacatgaagccattgtgaagaatgtacatgatctgctagcaaagttggcttgggatttttctcctggacaacttgatcatctttttgattgctttaaggcaagttggacaaatgcaagtaaaaagcaacgtgaaaagctccttgagttgatacgccgtcttgcagaagatgataaagatggtgtgatggcacacaaagtgttgaaccttctttggaacctggctcagagtgatgatgtgcctgtatacatcatggaccttgctcttagtgcccacataaaaatactagattatagttgtgcccaggatcgagatgcacagaagatccagtggatagatcactttatagaagaacttcgcacaaatgacaagtgggtaattcctgctctgaaacaaataagagaaatttgtagtttgtttggtgaagcatctcaaaatttgagtcaaactcagcgaagtccccacatattttatcgccatgatttaatcaaccagcttcaacaaaatcatgctttagttactttggtagcagaaaaccttgcaacctacatgaatagcatcagattgtatgctggagatcatgaagactatgatccacaaacagtgaggcttggaagtcgatacagtcatgttcaagaagttcaagaacgactaaacttccttagatttttagtgaaggatggccaactgtggctctgtgctcctcaggcaaaacaaatatggaagtgcttagcagaaaatgcagtttatctttgtgatcgtgaagcctgttttaagtggtattccaagttaatgggggatgaaccagacttggatcctgatattaataaggacttctttgaaagtaatgtacttcagcttgatccttcccttttaactgaaaatggaatgaaatgctttgaaagatttttcaaagctgtcaattgtcgagaaaggaaactaatagcaaaaagaagatcctatatgatggatgatttggaattaattggactagactacctttggagggttgtgattcagagtagtgacgagattgctaacagagctatagatcttcttaaagagatatacacaaaccttggcccaagattaaaagccaatcaggtggttatccatgaagacttcattcagtcttgctttgatcgtttaaaagcatcatatgatacactgtgtgtttttgatggtgacaaaaacagcattaattgtgcaagacaagaagccattcgaatggttagagtattaactgttataaaagagtacattaatgaatgtgacagtgattatcacaaggaaagaatgattctacctatgtcgagagcatttcgtggcaaacacctctctcttatagttcggtttccaaaccagggcagacaggttgatgagttggatatatggtctcatacgaatgacacaattggttcagtacggcgatgtattgttaatcgtattaaagccaatgtagcccacaaaaaaattgaactttttgtgggtggtgagctgatagattctgaagatgacagaaagctaattggacaattaaacttaaaagataaatctctaattacagccaaacttacacaaataaatttcaatatgccatcaagtcctgatagctcttccgattcctcaactgcatctcctggaaaccaccgtaatcattacaatgatggtcccaatctagaggtggaaagttgtttgcctggggtgataatgtcagtgcatcccagatacatctctttcctttggcaagttgcagacttaggtagcaacctgaatatgccacctcttagagatggagcaagagtacttatgaaacttatgccaccagatagaacagctgtagaaaaattacgagctgtttgtttggaccatgcaaaacttggagaaggcaaacttagtccaccccttgactctcttttctttggtccttctgcctcccaagttctatacctaacagaggtagtttatgccttgttaatgcctgctggtgtgcctctaactgatgggtcctctgactttcaagttcacttcttgaaaagtggtggcttacctcttgtactgagtatgctaataagaaataacttcttgccaaatacagatatggaaactcgaaggggtgcttatttaaatgctcttaaaatagccaaactgttgttaactgcgattggctatggccatgttcgagctgtagcagaagcttgtcagccagttgtagatggtacagaccccataacacagattaaccaagttactcatgatcaagcagtggtgctacaaagtgcccttcagagcattcctaatccctcatccgagtgcgtacttagaaatgagtccatacttcttgctcaggaaatatctaatgaggcttcaagatatatgcctgatatttgtgtaattagggctatacagaaaattatctgggcatcagcatgtggggcattaggactagtttttagcccaaatgaagaaataactaaaatttatcagatgaccaccaatggaagcaataagctggaggtggaagatgaacaagtttgctgtgaagcactggaagtgatgaccttatgttttgctttacttccaacagcgttggatgcacttagtaaagaaaaagcctggcagaccttcatcattgacttattattgcactgtccaagcaaaactgttcgtcagttggcacaggagcagttctttttaatgtgcaccagatgttgcatgggacacaggcctctgcttttcttcattactttactctttaccatactggggagcacagcaagagagaagggtaaatattcaggtgattatttcacacttttacggcaccttctcaattatgcttacaatggcaatattaacatacccaatgctgaagttcttcttgtcagtgaaattgattggctcaaaaggattagggataatgttaaaaacacaggtgaaacaggtgtcgaagagccaatactggaaggccaccttggggtaacaaaagagttattggcctttcaaacttctgagaaaaagtatcactttggttgtgaaaaaggaggtgctaatctcattaaagaattaattgatgatttcatctttcccgcatccaaagtttacctgcagtatttaagaagtggagaactaccagctgagcaggctattccagtctgtagttcacccgttaccatcaatgccggttttgagctacttgtagcattagctattggctgtgtgaggaatctcaaacagatagtagactgtttgactgaaatgtattacatgggcacagcaattactacttgtgaagcacttactgagtgggaatatctgccccctgttggaccccgcccaccaaaaggatttgtgggactcaaaaatgctggtgctacgtgttacatgaactctgtgatccagcagctatacatgattccttctatcaggaacagtattcttgcaattgaaggcacaggtagtgatttacacgatgatatgttcggggatgagaagcaggacagtgagagtaatgttgatccccgagatgatgtatttggatatcctcatcaatttgaagacaagccagcattaagtaagacagaagataggaaagagtataatattggtgtcctaagacaccttcaggtcatctttggtcatttagctgcttcccaactacaatactatgtacccagaggattttggaaacagttcaggctttggggtgaacctgttaatctccgtgaacaacatgatgccttagagttttttaattctttggtggatagtttagatgaagctttaaaagctttaggacacccggctatactaagtaaagtcctaggaggctcctttgctgatcagaagatctgccaaggctgcccacataggtatgaatgtgaagaatcttttacaactttgaatgtggatattagaaatcatcaaaatcttcttgactctttggaacagtatatcaaaggagatttattggaaggtgcaaatgcatatcattgtgaaaaatgtgataaaaaggttgacacagtaaagcgcctgctaattaaaaaattgcctcgggttcttgctatccaactcaaacgatttgactatgactgggaaagagaatgtgcaattaaattcaatgattattttgaatttcctcgagagctggatatgggaccttacacagtagcaggtgttgcaaacctggaaagggataatgtaaactcagaaaatgagttgattgaacagaaagagcagtctgacaatgaaactgcaggaggcacaaagtacagacttgtaggagtgcttgtacacagtggtcaagcaagcggtgggcattattattcttacatcattcaaaggaatggtaaagatgatcagacagatcactggtataaatttgatgatggagatgtaacagaatgcaaaatggatgatgatgaagaaatgaaaaatcagtgttttggtggagagtacatgggagaagtatttgatcacatgatgaagcgcatgtcatataggcgacagaagaggtggtggaatgcttacatacttttttatgaacaaatggatatgatagatgaagatgatgagatgataagatacatatcagagctaactattgcaagaccccatcagatcattatgtcaccagccattgagagaagtgtacggaaacaaaatgtgaaatttatgcataaccgattgcaatatagtttagagtattttcagtttgtgaaaaaactgcttacatgtaatggtgtttatttaaaccctgctccagggcaggattatttgttgcctgaagcagaagaaattactatgattagtattcagcttgctgctagattcctctttaccactggatttcacaccaagaaaatagttcgtggtcctgccagtgactggtatgatgcactgtgcgttcttctccgtcacagcaaaaatgtaggtttttggtttactcataatgtcctttttaatgtatcaaatcgcttctctgaataccttctggagtgccctagtgcagaagtgaggggtgcatttgcaaaacttatagtgtttattgcacacttttccttgcaagatgggtcttgtccttctccttttgcatctccaggaccttctagtcaggcatgtgataacttgagcttgagtgaccacttactaagagccacactaaatctcttgagaagggaagtttcagagcatggacatcatttacagcaatattttaatttgtttgtaatgtatgccaatttaggtgtggcagaaaaaacacagcttctgaaattgaatgtacctgctacctttatgcttgtgtctttagacgaaggaccaggtcctccaatcaaatatcagtatgctgaattaggcaagttatattcagtagtgtctcagctgattcgttgttgcaatgtgtcatcaacaatgcagtcttcaatcaatggtaatccccctctccccaatcctttcggtgaccttaatttatcacagcctataatgccaattcagcagaatgtgttagacattttatttgtgagaacaagttatgtgaagaaaattattgaagactgcagtaactcagaggataccatcaaattacttcgcttttgctcttgggagaatcctcagttctcatctactgtcctcagcgaacttctctggcaggttgcatattcatatacctatgaacttcggccatatttagatctacttttccaaattttactgattgaggactcctggcagactcacagaattcataatgcacttaaaggaattccagatgacagagatgggctgttcgatacaatacagcgctcgaagaatcactatcaaaaacgagcatatcagtgcataaaatgtatggtagctctatttagcagttgtcctgttgcttaccagatcttacagggtaacggagatcttaaaagaaaatggacctgggcagtggaatggctaggagatgaacttgaaagaagaccatatactggcaatcctcagtatagttacaacaattggtctcctccagtacaaagcaatgaaacagcaaatggttatttcttagaaagatcacatagtgctaggatgacacttgcaaaagcttgtgaactctgtccagaagaggagccagatgaccaggatgccccagatgagcatgagccctctccatcagaagatgccccattatatcctcattcacctgcctctcagtatcaacagaataatcatgtacatggacagccatatacaggaccagcagcacatcacttgaacaaccctcagaaaacaggccaacgaacacaagaaaattatgaaggcaatgaagaagtatcctcacctcagatgaaggatcagtgaaaagcaataattaactgcttcctttatgactatgcactaaggtcttatagtccaaactttctctgtgtctggctagtattgaaaactagataaactgctccaaaccaacatggagtaaagagcatattcactggtttatttgcagtaatttgcaatttgtcagtgtataagacacatgcagggtgaagtgtacagagttttgtaacaaatgactggtcctaatctgtaaatgagaaaggtatatatactatgttaatgtctgactgttaattcttaagcaagaaactttttttgatgaaaacaagtcagatctacacagtcacacaattattttttgttgtgttcactacattgtgcaattgatattgcctgctttgagcagtttggtcaacttaccaacttccccccaaaaaagggaacataaaagagcccatctttgtcagtttacaccaatagtttcttgttaatccttctttcctggatatataaggctggtggtaacttttgaattatatggttgatgtggaaaattggcagtgtaacatttctagatacttttcattacctttttattctggtatataggctaaccactttaaagctattcttatgctgtaacagttagcatggcttcacactgtttgtgtagccaagaggacagaattacatgaatgacagtgcccagagtgacagctgtatattgctcagagcttttatttcttatacctagaataaatataaaatgggggaaaaaaaaaa

SEQ ID NO: 16 - RNA, 1143 nt, Homo sapiens
  source 1..1143: mol_type = other RNA
aatcgtcaatgcgacgtcctcctactcccacctcagagctgtcacagagactgtcagttccgtccctccccttcagccctttaacgcacgtcttcccgaccgcataacttgctcagtccctgcggccaactggggcgggccaatggctgtgacggataaggggtgtggggtgcggggacaatgggccagagcttctcatgcagcctgcaccagcgccgggtcggagagtcagaggccaccctgagatggaccgagatcttcagttggggaggcgcctccggtgagcttgcggccagatgccccctcagtagtcctccgcaacaggtgccgcgcagccgagtggcgggctagcataccgcctgcccgcaattcggccaggcctcgagcctgctccgccttcccgctgcggtagcgccgccggggaaacgccgccacgggctgcatgggcagcgctcgcgccccgccgctgagccgccggggagccgtccagtcttcgaatcccagaaacacaaagatggtgcagacccaggccctgctttgactgggagaaagatgcattcagttgactaaaacttgaaaactgtccatttggctatgagcgaatcatcctgcttgcttttataagcatttatcctgaaaagaaatttaaagcagacatcccataaatggagtctgggacagaaacctacacattggggcttggtggcatgcatgtttagtcccagctacacagcagggaggctgaggctgaaggaatacttgagcccaggaattcaagactagcctgcacaacatatttcaggtggagcctctgggaggtgatgaggtcatgagagtggagcctcatgaatgggatgagcactcctacaaaaaggattccagagagctcgcttgctccttccacagtgtgaggacacagagggaaggctctgtctatgaatgagaaagtgggtccccaccagacattgaatctgccgcatcttgatactggacttccagtctccagaactgtgggcaataaatgtctgttgtttattacctgtccagtatctttggtattttgctatagcaacccaaatggactaagaaaacaccagaggccatacctaataaaaatattgacatcacaaaaaaaaaaaaaaa

SEQ ID NO: 17 - RNA, 1063 nt, Homo sapiens
  source 1..1063: mol_type = other RNA
aatcgtcaatgcgacgtcctcctactcccacctcagagctgtcacagagactgtcagttccgtccctccccttcagccctttaacgcacgtcttcccgaccgcataacttgctcagtccctgcggccaactggggcgggccaatggctgtgacggataaggggtgtggggtgcggggacaatgggccagagcttctcatgcagcctgcaccagcgccgggtcggagagtcagaggccaccctgagatggaccgagatcttcagttggggaggcgcctccggtgagcttgcggccagatgccccctcagtagtcctccgcaacaggtgccgcgcagccgagtggcgggctagcataccgcctgcccgcaattcggccaggcctcgagcctgctccgccttcccgctgcggtagcgccgccggggaaacgccgccacgggctgcatgggcagcgctcgcgccccgccgctgagccgccggggagccgtccagtcttcgaatcccagaaacacaaagatggtgcagacccaggccctgctttgactgggagaaagatgcattcagttgactaaaacttgaaccacagcatgttccgaagagatgattggaagatggaagtggagggttaaataatgaaatgcagctaacatttcggaaagtttctaaaagttgtacaacatgccctacagctactctttaaatctccaaatcaaatgagtttcaggtggagcctctgggaggtgatgaggtcatgagagtggagcctcatgaatgggatgagcactcctacaaaaaggattccagagagctcgcttgctccttccacagtgtgaggacacagagggaaggctctgtctatgaatgagaaagtgggtccccaccagacattgaatctgccgcatcttgatactggacttccagtctccagaactgtgggcaataaatgtctgttgtttattacctgtccagtatctttggtattttgctatagcaacccaaatggactaagaaaacaccagaggccatacctaataaaaatattgacatcacaaaaaaaaaaaaaaa

SEQ ID NO: 18 - RNA, 988 nt, Homo sapiens
  source 1..988: mol_type = other RNA
aatcgtcaatgcgacgtcctcctactcccacctcagagctgtcacagagactgtcagttccgtccctccccttcagccctttaacgcacgtcttcccgaccgcataacttgctcagtccctgcggccaactggggcgggccaatggctgtgacggataaggggtgtggggtgcggggacaatgggccagagcttctcatgcagcctgcaccagcgccgggtcggagagtcagaggccaccctgagatggaccgagatcttcagttggggaggcgcctccggtgagcttgcggccagatgccccctcagtagtcctccgcaacaggtgccgcgcagccgagtggcgggctagcataccgcctgcccgcaattcggccaggcctcgagcctgctccgccttcccgctgcggtagcgccgccggggaaacgccgccacgggctgcatgggcagcgctcgcgccccgccgctgagccgccggggagccgtccagtcttcgaatcccaccacagcatgttccgaagagatgattggaagatggaagtggagggttaaataatgaaatgcagctaacatttcggaaagtttctaaaagttgtacaacatgccctacagctactctttaaatctccaaatcaaatgagtttcaggtggagcctctgggaggtgatgaggtcatgagagtggagcctcatgaatgggatgagcactcctacaaaaaggattccagagagctcgcttgctccttccacagtgtgaggacacagagggaaggctctgtctatgaatgagaaagtgggtccccaccagacattgaatctgccgcatcttgatactggacttccagtctccagaactgtgggcaataaatgtctgttgtttattacctgtccagtatctttggtattttgctatagcaacccaaatggactaagaaaacaccagaggccatacctaataaaaatattgacatcacaaaaaaaaaaaaaaa

SEQ ID NO: 19 - RNA, 738 nt, Homo sapiens
  source 1..738: mol_type = other RNA
gagttgggaggaaagcggcggcggtggcggcttcaacagcagctcttgcccttaaggaacaatgaaacacaaagatggtgcagacccaggccctgctttgactgggagaaagatgcattcagttgactaaaacttgaaagatgtttgaaatacaacaaaatagttggaagaatctcccaacacagttggaagactatctactggggagaagtgttcagtatcataaagataacatctcatccagaggaaagtgccacagcatgttccgaagagatgattggaagatggaagtggagggttaaataatgaaatgcagctaacatttcggaaagtttctaaaagttgtacaacatgccctacagctactctttaaatctccaaatcaaatgagtttcaggtggagcctctgggaggtgatgaggtcatgagagtggagcctcatgaatgggatgagcactcctacaaaaaggattccagagagctcgcttgctccttccacagtgtgaggacacagagggaaggctctgtctatgaatgagaaagtgggtccccaccagacattgaatctgccgcatcttgatactggacttccagtctccagaactgtgggcaataaatgtctgttgtttattacctgtccagtatctttggtattttgctatagcaacccaaatggactaagaaaacaccagaggccatacctaataaaaatattgacatcacaaaaaaaaaaaaaaa

SEQ ID NO: 20 - RNA, 901 nt, Homo sapiens
  source 1..901: mol_type = other RNA
aatcgtcaatgcgacgtcctcctactcccacctcagagctgtcacagagactgtcagttccgtccctccccttcagccctttaacgcacgtcttcccgaccgcataacttgctcagtccctgcggccaactggggcgggccaatggctgtgacggataaggggtgtggggtgcggggacaatgggccagagcttctcatgcagcctgcaccagcgccgggtcggagagtcagaggccaccctgagatggaccgagatcttcagttggggaggcgcctccggtgagcttgcggccagatgccccctcagtagtcctccgcaacaggtgccgcgcagccgagtggcgggctagcataccgcctgcccgcaattcggccaggcctcgagcctgctccgccttcccgctgcggtagcgccgccggggaaacgccgccacgggctgcatgggcagcgctcgcgccccgccgctgagccgccggggagccgtccagtcttcgaatcccagcttggtggcatgcatgtttagtcccagctacacagcagggaggctgaggctgaaggaatacttgagcccaggaattcaagactagcctgcacaacatagtgagaccctgactttaaaataaatttaaaaaaattaaaagcaacaagactttctgcttgtatatgatgatgttagtatgctgacttacaaggttagatcattttgatatgtgtgatgtaggttttcaaagctggcactgttttatgcttcaaatattatttttattcattggttctcatgggatttcatcactaagctgtaaatcaataatcataatgttgaggggaggggattacaaaatagctcttcaaaatcatctttgcatttctcaataaacagcattcccttttgaaaaaaa

SEQ ID NO: 21 - RNA, 536 nt, Homo sapiens
  source 1..536: mol_type = other RNA
gagttgggaggaaagcggcggcggtggcggcttcaacagcagctcttgcccttaaggaacaatgaaacacaaagatggtgcagacccaggccctgctttgactgggagaaagatgcattcagttgactaaaacttgaagcttggtggcatgcatgtttagtcccagctacacagcagggaggctgaggctgaaggaatacttgagcccaggaattcaagactagcctgcacaacatagtgagaccctgactttaaaataaatttaaaaaaattaaaagcaacaagactttctgcttgtatatgatgatgttagtatgctgacttacaaggttagatcattttgatatgtgtgatgtaggttttcaaagctggcactgttttatgcttcaaatattatttttattcattggttctcatgggatttcatcactaagctgtaaatcaataatcataatgttgaggggaggggattacaaaatagctcttcaaaatcatctttgcatttctcaataaacagcattcccttttgaaaaaaa

SEQ ID NO: 22 - RNA, 624 nt, Homo sapiens
  source 1..624: mol_type = other RNA
ggggagggtaggcaggtcggaggagggagttgggaggaaagcggcggcggtggcggcttcaacagcagctcttgcccttaaggaacaatgcctccagtcggatcctgcgtcattctggctgccttggcctttcctttcctcagttgagccagccacagcatgttccgaagagatgattggaagatggaagtggagggttaaataatgaaatgcagctaacatttcggaaagtttctaaaagttgtacaacatgccctacagctactctttaaatctccaaatcaaatgagtttcaggtggagcctctgggaggtgatgaggtcatgagagtggagcctcatgaatgggatgagcactcctacaaaaaggattccagagagctcgcttgctccttccacagtgtgaggacacagagggaaggctctgtctatgaatgagaaagtgggtccccaccagacattgaatctgccgcatcttgatactggacttccagtctccagaactgtgggcaataaatgtctgttgtttattacctgtccagtatctttggtattttgctatagcaacccaaatggactaagaaaacaccagaggccatacctaataaaaatattgacatcacaa

SEQ ID NO: 23 - RNA, 1203 nt, Homo sapiens
  source 1..1203: mol_type = other RNA
ggggagggtaggcaggtcggaggagggagttgggaggaaagcggcggcggtggcggcttcaacagcagctcttgcccttaaggaacaatgaaacacaaagatggtgcagacccaggccctgctttgactgggagaaagatgcattcagttgactaaaacttgaacagggcagtttacttctatagaagggtgcaccctcacagatggaccaatgtgtcaggagaattcagtcacacccaaagcaggaggtaataagacaccgaagtgaggacttcacaggctgcttgggagaagacaatcatccgtgggcttgggaaagggagaaatgcctactgagtttagggaattgcttgctggaagaaatgatggcttggtggcatgcatgtttagtcccagctacacagcagggaggctgaggctgaaggaatacttgagcccaggaattcaagactagcctgcacaacatagtgagaccctgactttaaaataaatttaaaaaaattaaaagcaacaagactttctgcttgtatatgatgatgttagtatgctgacttacaaggttagatcattttgatatgtgtgatgtaggttttcaaagctggcactgttttatgcttcaaatattatttttattcattggttctcatgggatttcatcactaagctgtaaatcaataatcataatgttgaggggaggggattacaaaatagctcttcaaaatcatctttgcatttctcaataaacagcattcccttttggactacagtgaaaaatattgagctttgtttactttgaaaatgagtcttagtctatgaatgcctgggtagggtcaagaatgaaaaatgagaggaagagagaagcatcaggaagataaaatgatcaatctcacaaaacttgctatttttagaaagcatcattctaattttgaaaccaaaaaaatggggaaaaacagagtaatggaataatagaatgcctcatgtacaaaagcaacaatttcagagatgatctaaaacaacttattagttataggaagaaatatacctgaaaagggcaaaaataagttgggtttggcctcttgtcactgaaattatctactaaatctaacagcatctatgttcctttagctgttgtgtatattgtacacaaatgtgaaaccataactcatattttacctataacaatttgcaataaataactaatta

SEQ ID NO: 24 - RNA, 537 nt, Homo sapiens
  source 1..537: mol_type = other RNA
tggtgagccagccaggagtgaagacgacaggtttgctgtctcctttgcctgtgggtctggggccccagcctgggggagacccgtgactccaggcatgctatcaggacaacttcaacccgaggggagatcagctctcccgcaacctggtgccgctctctgacagcacaacagaacctaaggggctacaggatgattcaaggaacagtgtgctacaggacctcgcaagaagaccctcaccagatgcagcccctctatgttggacttcccagcctccggaagttagaaatgtgctacaaccactcaaggtctgcaaacagattcctatttagatgttgttgagagctgaatttctggaacaagagatatagattaagactgttgttacatgttgcctacatgactttcaaaagcttgattcccagtggcgctctcaacagcagtcataaacaatggtaattcaatgtatatttatattcaactgatatattaattggaatatattaaaaatacgtatatttatattcagaataaaaaaaa

SEQ ID NO: 25 - RNA, 537 nt, Homo sapiens; identical to SEQ ID NO: 24
  source 1..537: mol_type = other RNA

SEQ ID NO: 26 - RNA, 901 nt, Homo sapiens; identical to SEQ ID NO: 20
  source 1..901: mol_type = other RNA

SEQ ID NO: 27 - RNA, 2175 nt, Homo sapiens
  source 1..2175: mol_type = other RNA
atggatggtgatcagattgttgtggaaatacaagaagcagtttttgtttctaatattgtggattctgacataactgtgcataactttgttcctgatgacccagactcagttgtaatccaagatgttgttgaagatgttgtcatagaggaggatgttcagtgctcagatatcttagaagaggcagatgtatctgaaaatgtcatcattcctgagcaagtgctggactcagatgtaactgaagaagtttctttaccacactgcacagtcccagatgatgttttagcttctgacattacttcaacctcaatgtctatgccagaacatgttttaacgagtgaatccatgcatgtgtgtgacattggacatgttgaacatatggtgcatgatagtgtagtggaagcagaaatcattactgatcctctgacgagtgacatagtttcagaagaagtattggtagcagactgtgcccctgaagcagtcatagatgccagcgggatctcagtggaccagcaagataatgacaaagccagctgtgaggactacctaatgatttcgttggatgatgctggcaaaatagaacatgatggttccactggagtgaccatcgatgcagaatcagaaatggatccttgtaaagtggatagcacttgtcctgaagtcatcaaggtgtacatttttaaagctgaccctggagaagatgacttaggtggaactgtagacattgtggagagtgaacctgaaaatgatcatggagttgaactacttgatcagaacagcagtattcgtgttcccagggaaaagatggtttatatgactgtcaatgactctcaacaagaagatgaagatttaagtaataattctgatggaattgaaaaccggaatggcactgcaagtgccctcttgcacatagatgagtctgctggccttggcagactggctaaacagaaaccaaagaaaaagagaagacctgattccaggcagtaccaaacagcaataattattggccctgatggtcatcctttgactgtctatccttgcatgatttgtgggaagaagtttaagtcgaggggttttttgaaaagacacatgaaaaaccatcctgaacaccttgccaagaagaagtaccactgtactgactgtgattacactaccaataagaagataagtttacataaccacctggagagccacaagctgaccagcaaggcagagaaggccattgaatgtgatgagtgtgggaagcatttttctcatgcaggggctttgtttactcacaaaatggtgcataaggaaaaaggggccaacaaaatgcacaagtgtaaattctgtgaatatgagacagctgaacaggggttattgaatcgccacctcttggcagtccacagcaagaactttcctcatatttgtgtggagtgtggtaaaggtttccgacacccgtcggaactgagaaagcacatgcgaatccataccggcgagaagccataccaatgccagtactgtgaatataggtctgcagactcttctaacttgaaaacacatataaaaacaaagcatagtaaagagatgccattcaagtgtgacatttgtcttctgactttctcagataccaaagaagtgcagcaacatactcttgtccaccaagaaagcaaaacacatcagtgtttgcattgcgaccacaagagttcaaactcaagtgatttgaaacgacatgtaatttcagttcatacgaaagactatcctcataagtgtgagatgtgcgagaaaggctttcacaggccttcagaacttaagaaacatgtggctgtccacaaaggtaaaaaaatgcaccaatgtagacattgtgactttaagattgcagacccatttgttctaagtcgccatattctctcagttcacacaaaggatcttccatttaggtgtaagagatgtagaaagggatttaggcaacaaaatgagcttaaaaagcatatgaagacacacagtggcaggaaagtatatcagtgtgagtactgtgagtatagcactacagatgcctcaggctttaaacggcacgttatttccattcatacaaaagactatcctcatcggtgtgagtactgcaagaaaggcttccgaagaccttcagaaaagaaccagcacataatgagacaccataaagaagttggtctgccctaa

SEQ ID NO: 28 - DNA, 20 bp, Homo sapiens
  source 1..20: mol_type = other DNA
ggcgacctggaagtccaact

SEQ ID NO: 29 - DNA, 20 bp, Homo sapiens
  source 1..20: mol_type = other DNA
ccatcagcaccacagccttc

SEQ ID NO: 30 - DNA, 23 bp, Homo sapiens
  source 1..23: mol_type = other DNA
tgaggaagattactgtgggagtg

SEQ ID NO: 31 - DNA, 24 bp, Homo sapiens
  source 1..24: mol_type = other DNA
aatcaccatacacaaattgcctgt

SEQ ID NO: 32 - DNA, 22 bp, Homo sapiens
  source 1..22: mol_type = other DNA
aagcttgtcaaagggatgagtc

SEQ ID NO: 33 - DNA, 23 bp, Homo sapiens
  source 1..23: mol_type = other DNA
tcagagttcaggtccagattagc

SEQ ID NO: 34 - DNA, 23 bp, Homo sapiens
  source 1..23: mol_type = other DNA
catctccaggaccaaatgtgtct

SEQ ID NO: 35 - DNA, 23 bp, Homo sapiens
  source 1..23: mol_type = other DNA
ggaagcattgtgttttgatggtg

SEQ ID NO: 36 - DNA, 23 bp, Homo sapiens
  source 1..23: mol_type = other DNA
agcagttgtcctgttgcttacca

SEQ ID NO: 37 - DNA, 21 bp, Homo sapiens
  source 1..21: mol_type = other DNA
ggggcatcttctgatggagag

SEQ ID NO: 38 - DNA, 17 bp, Homo sapiens
  source 1..17: mol_type = other DNA
gcaggcgtgaggagctg

SEQ ID NO: 39 - DNA, 20 bp, Homo sapiens
  source 1..20: mol_type = other DNA
ggctcttgtggctgcaattc

SEQ ID NO: 40 - DNA, 23 bp, Homo sapiens
  source 1..23: mol_type = other DNA
tgtgcacgaaaaacaagcaaaag

SEQ ID NO: 41 - DNA, 25 bp, Homo sapiens
  source 1..25: mol_type = other DNA
aggatgataatgaaagagctagtgt

SEQ ID NO: 42 - DNA, 21 bp, Homo sapiens
  source 1..21: mol_type = other DNA
ctacaaccactcaaggtctgc

SEQ ID NO: 43 - DNA, 20 bp, Homo sapiens
  source 1..20: mol_type = other DNA
tatgactgctgttgagagcg

SEQ ID NO: 44 - DNA, 20 bp, Homo sapiens
  source 1..20: mol_type = other DNA
gtgacggataaggggtgtgg

SEQ ID NO: 45 - DNA, 20 bp, Homo sapiens
  source 1..20: mol_type = other DNA
atctcggtccatctcagggt

SEQ ID NO: 46 - DNA, 19 bp, Homo sapiens
  source 1..19: mol_type = other DNA
ttactcctcgcgtccaaag

SEQ ID NO: 47 - DNA, 20 bp, Homo sapiens
  source 1..20: mol_type = other DNA
acgatccttgcagatggctt

SEQ ID NO: 48 - DNA, 20 bp, Rattus norvegicus
  source 1..20: mol_type = other DNA
cccgtatacagtgcggtgtc

SEQ ID NO: 49 - DNA, 19 bp, Rattus norvegicus
  source 1..19: mol_type = other DNA
tcaatcctaccccgaagca

SEQ ID NO: 50 - DNA, 20 bp, Rattus norvegicus
  source 1..20: mol_type = other DNA
gcaccgcaaatgcttctagg

SEQ ID NO: 51 - DNA, 20 bp, Rattus norvegicus
  source 1..20: mol_type = other DNA
cgatggtcgattgtcgtcct

SEQ ID NO: 52 - DNA, 21 bp, Rattus norvegicus
  source 1..21: mol_type = other DNA
tctctgctcctccctgttcta

SEQ ID NO: 53 - DNA, 20 bp, Rattus norvegicus
  source 1..20: mol_type = other DNA
atgaaggggtcgttgatggc